European Patent Application EP 4 574 162 A2, published June 25, 2025. Title: BONE MORPHOGENETIC PROTEIN-9 AND -10 VARIANTS WITH ENHANCED THERAPEUTIC EFFECT DUE TO REDUCED SIDE EFFECTS OF ECTOPIC OSSIFICATION AND PHARMACEUTICAL COMPOSITION COMPRISING SAME. Applicant: NIBEC Co., Ltd. Application EP. The sequence listing filed with the application follows.

SEQUENCE LISTING (34 sequences)

SEQ ID NO: 1 - protein, 426 aa, Homo sapiens
MAWVWTLLFLMAAAQSIQAKPLQSWGRGSAGGNAHSPLGVPGGGLPEHTFNLKMFLENVKVDFLRSLNLSGVPSQDKTRVEPPQYMIDLYNRYTSDKSTTPASNIVRSFSMEDAISITATEDFPFQKHILLFNISIPRHEQITRAELRLYVSCQNHVDPSHDLKGSVVIYDVLDGTDAWDSATETKTFLVSQDIQDEGWETLEVSSAVKRWVRSDSTKSKNKLEVTVESHRKGCDTLDISVPPGSRNLPFFVVFSNDHSSGTKETRLELREMISHEQESVLKKLSKDGSTEAGESSHEEDTDGHVAAGSTLARRKRSAGAGSHCQKTSLRVNFEDIGWDSWIIAPKEYEAYECKGGCFFPLADDVTPTKHAIVQTLVHLKFPTKVGKACCVPTKLSPISVLYKDDMGVPTLKYHYEGMSVAECGCR

SEQ ID NO: 2 - protein, 426 aa, synthetic construct
  source 1..426: note = BMP-9 varient
MAWVWTLLFLMAAAQSIQAKPLQSWGRGSAGGNAHSPLGVPGGGLPEHTFNLKMFLENVKVDFLRSLNLSGVPSQDKTRVEPPQYMIDLYNRYTSDKSTTPASNIVRSFSMEDAISITATEDFPFQKHILLFNISIPRHEQITRAELRLYVSCQNHVDPSHDLKGSVVIYDVLDGTDAWDSATETKTFLVSQDIQDEGWETLEVSSAVKRWVRSDSTKSKNKLEVTVESHRKGCDTLDISVPPGSRNLPFFVVFSNDHSSGTKETRLELREMISHEQESVLKKLSKDGSTEAGESSHEEDTDGHVAAGSTLARRKRSAGAGSHCQKTSLRVNFEAIGWDSWIIAPKEYEAYECKGGCFFPLADDVTPTKHAIVQTLVHLKFPTKVGKACCVPTKLSPISVLYKDDMGVPTLKYHYEGMSVAECGCR

SEQ ID NO: 3 - protein, 426 aa, synthetic construct
  source 1..426: note = BMP-9 varient
MAWVWTLLFLMAAAQSIQAKPLQSWGRGSAGGNAHSPLGVPGGGLPEHTFNLKMFLENVKVDFLRSLNLSGVPSQDKTRVEPPQYMIDLYNRYTSDKSTTPASNIVRSFSMEDAISITATEDFPFQKHILLFNISIPRHEQITRAELRLYVSCQNHVDPSHDLKGSVVIYDVLDGTDAWDSATETKTFLVSQDIQDEGWETLEVSSAVKRWVRSDSTKSKNKLEVTVESHRKGCDTLDISVPPGSRNLPFFVVFSNDHSSGTKETRLELREMISHEQESVLKKLSKDGSTEAGESSHEEDTDGHVAAGSTLARRKRSAGAGSHCQKTSLRVNFEDIEWDSWIIAPKEYEAYECKGGCFFPLADDVTPTKHAIVQTLVHLKFPTKVGKACCVPTKLSPISVLYKDDMGVPTLKYHYEGMSVAECGCR

SEQ ID NO: 4 - protein, 426 aa, synthetic construct
  source 1..426: note = BMP-9 varient
MAWVWTLLFLMAAAQSIQAKPLQSWGRGSAGGNAHSPLGVPGGGLPEHTFNLKMFLENVKVDFLRSLNLSGVPSQDKTRVEPPQYMIDLYNRYTSDKSTTPASNIVRSFSMEDAISITATEDFPFQKHILLFNISIPRHEQITRAELRLYVSCQNHVDPSHDLKGSVVIYDVLDGTDAWDSATETKTFLVSQDIQDEGWETLEVSSAVKRWVRSDSTKSKNKLEVTVESHRKGCDTLDISVPPGSRNLPFFVVFSNDHSSGTKETRLELREMISHEQESVLKKLSKDGSTEAGESSHEEDTDGHVAAGSTLARRKRSAGAGSHCQKTSLRVNFEDIGWDSWIIAPKEYEAYECKGGCFFPLADEVTPTKHAIVQTLVHLKFPTKVGKACCVPTKLSPISVLYKDDMGVPTLKYHYEGMSVAECGCR

SEQ ID NO: 5 - protein, 426 aa, synthetic construct
  source 1..426: note = BMP-9 varient
MAWVWTLLFLMAAAQSIQAKPLQSWGRGSAGGNAHSPLGVPGGGLPEHTFNLKMFLENVKVDFLRSLNLSGVPSQDKTRVEPPQYMIDLYNRYTSDKSTTPASNIVRSFSMEDAISITATEDFPFQKHILLFNISIPRHEQITRAELRLYVSCQNHVDPSHDLKGSVVIYDVLDGTDAWDSATETKTFLVSQDIQDEGWETLEVSSAVKRWVRSDSTKSKNKLEVTVESHRKGCDTLDISVPPGSRNLPFFVVFSNDHSSGTKETRLELREMISHEQESVLKKLSKDGSTEAGESSHEEDTDGHVAAGSTLARRKRSAGAGSHCQKTSLRVNFEDIGWDSWIIAPKEYEAYECKGGCFFPLADDVTPTKHDIVQTLVHLKFPTKVGKACCVPTKLSPISVLYKDDMGVPTLKYHYEGMSVAECGCR

SEQ ID NO: 6 - protein, 426 aa, synthetic construct
  source 1..426: note = BMP-9 varient
MAWVWTLLFLMAAAQSIQAKPLQSWGRGSAGGNAHSPLGVPGGGLPEHTFNLKMFLENVKVDFLRSLNLSGVPSQDKTRVEPPQYMIDLYNRYTSDKSTTPASNIVRSFSMEDAISITATEDFPFQKHILLFNISIPRHEQITRAELRLYVSCQNHVDPSHDLKGSVVIYDVLDGTDAWDSATETKTFLVSQDIQDEGWETLEVSSAVKRWVRSDSTKSKNKLEVTVESHRKGCDTLDISVPPGSRNLPFFVVFSNDHSSGTKETRLELREMISHEQESVLKKLSKDGSTEAGESSHEEDTDGHVAAGSTLARRKRSAGAGSHCQKTSLRVNFEDIGWDSWIIAPKEYEAYECKGGCFFPLADDVTPTKHAIVQTLVHLKFPTKVGKACCVPTKLSPISVLYKDEMGVPTLKYHYEGMSVAECGCR

SEQ ID NO: 7 - protein, 426 aa, synthetic construct
  source 1..426: note = BMP-9 varient
MAWVWTLLFLMAAAQSIQAKPLQSWGRGSAGGNAHSPLGVPGGGLPEHTFNLKMFLENVKVDFLRSLNLSGVPSQDKTRVEPPQYMIDLYNRYTSDKSTTPASNIVRSFSMEDAISITATEDFPFQKHILLFNISIPRHEQITRAELRLYVSCQNHVDPSHDLKGSVVIYDVLDGTDAWDSATETKTFLVSQDIQDEGWETLEVSSAVKRWVRSDSTKSKNKLEVTVESHRKGCDTLDISVPPGSRNLPFFVVFSNDHSSGTKETRLELREMISHEQESVLKKLSKDGSTEAGESSHEEDTDGHVAAGSTLARRKRSAGAGSHCQKTSLRVNFEDIGWDSWIIAPKEYEAYECKGGCFFPLADDVTPTKHAIVQTLVHLKFPTKVGKACCVPTKLSPISVLYKDNMGVPTLKYHYEGMSVAECGCR

SEQ ID NO: 8 - protein, 426 aa, synthetic construct
  source 1..426: note = BMP-9 varient
MAWVWTLLFLMAAAQSIQAKPLQSWGRGSAGGNAHSPLGVPGGGLPEHTFNLKMFLENVKVDFLRSLNLSGVPSQDKTRVEPPQYMIDLYNRYTSDKSTTPASNIVRSFSMEDAISITATEDFPFQKHILLFNISIPRHEQITRAELRLYVSCQNHVDPSHDLKGSVVIYDVLDGTDAWDSATETKTFLVSQDIQDEGWETLEVSSAVKRWVRSDSTKSKNKLEVTVESHRKGCDTLDISVPPGSRNLPFFVVFSNDHSSGTKETRLELREMISHEQESVLKKLSKDGSTEAGESSHEEDTDGHVAAGSTLARRKRSAGAGSHCQKTSLRVNFEDIGWDSWIIAPKEYEAYECKGGCFFPLADDVTPTKHAIVQTLVHLKFPTKVGKACCVPTKLSPISVLYKDQMGVPTLKYHYEGMSVAECGCR

SEQ ID NO: 9 - protein, 426 aa, synthetic construct
  source 1..426: note = BMP-9 varient
MAWVWTLLFLMAAAQSIQAKPLQSWGRGSAGGNAHSPLGVPGGGLPEHTFNLKMFLENVKVDFLRSLNLSGVPSQDKTRVEPPQYMIDLYNRYTSDKSTTPASNIVRSFSMEDAISITATEDFPFQKHILLFNISIPRHEQITRAELRLYVSCQNHVDPSHDLKGSVVIYDVLDGTDAWDSATETKTFLVSQDIQDEGWETLEVSSAVKRWVRSDSTKSKNKLEVTVESHRKGCDTLDISVPPGSRNLPFFVVFSNDHSSGTKETRLELREMISHEQESVLKKLSKDGSTEAGESSHEEDTDGHVAAGSTLARRKRSAGAGSHCQKTSLRVNFEDIGWDSWIIAPKEYEAYECKGGCFFPLADDVTPTKHAIVQTLVHLKFPTKVGKACCVPTKLSPISVLYKDDMGVPTLKYHWEGMSVAECGCR

SEQ ID NO: 10 - protein, 426 aa, synthetic construct
  source 1..426: note = BMP-9 varient
MAWVWTLLFLMAAAQSIQAKPLQSWGRGSAGGNAHSPLGVPGGGLPEHTFNLKMFLENVKVDFLRSLNLSGVPSQDKTRVEPPQYMIDLYNRYTSDKSTTPASNIVRSFSMEDAISITATEDFPFQKHILLFNISIPRHEQITRAELRLYVSCQNHVDPSHDLKGSVVIYDVLDGTDAWDSATETKTFLVSQDIQDEGWETLEVSSAVKRWVRSDSTKSKNKLEVTVESHRKGCDTLDISVPPGSRNLPFFVVFSNDHSSGTKETRLELREMISHEQESVLKKLSKDGSTEAGESSHEEDTDGHVAAGSTLARRKRSAGAGSHCQKTSLRVNFEDIGWDSWIIAPKEYEAYECKGGCFFPKADDVTPTKHAIVQTLVHLKFPTKVGKACCVPTKLSPISVLYKDDMGVPTLKYHYEGMSVAECGCR

SEQ ID NO: 11 - protein, 426 aa, synthetic construct
  source 1..426: note = BMP-9 varient
MAWVWTLLFLMAAAQSIQAKPLQSWGRGSAGGNAHSPLGVPGGGLPEHTFNLKMFLENVKVDFLRSLNLSGVPSQDKTRVEPPQYMIDLYNRYTSDKSTTPASNIVRSFSMEDAISITATEDFPFQKHILLFNISIPRHEQITRAELRLYVSCQNHVDPSHDLKGSVVIYDVLDGTDAWDSATETKTFLVSQDIQDEGWETLEVSSAVKRWVRSDSTKSKNKLEVTVESHRKGCDTLDISVPPGSRNLPFFVVFSNDHSSGTKETRLELREMISHEQESVLKKLSKDGSTEAGESSHEEDTDGHVAAGSTLARRKRSAGAGSHCQKTSLRVNFEDIGWDSWIIAPKEYEAYECKGGCFFPLANDVTPTKHAIVQTLVHLKFPTKVGKACCVPTKLSPISVLYKDDMGVPTLKYHYEGMSVAECGCR

SEQ ID NO: 12 - protein, 426 aa, synthetic construct
  source 1..426: note = BMP-9 varient
MAWVWTLLFLMAAAQSIQAKPLQSWGRGSAGGNAHSPLGVPGGGLPEHTFNLKMFLENVKVDFLRSLNLSGVPSQDKTRVEPPQYMIDLYNRYTSDKSTTPASNIVRSFSMEDAISITATEDFPFQKHILLFNISIPRHEQITRAELRLYVSCQNHVDPSHDLKGSVVIYDVLDGTDAWDSATETKTFLVSQDIQDEGWETLEVSSAVKRWVRSDSTKSKNKLEVTVESHRKGCDTLDISVPPGSRNLPFFVVFSNDHSSGTKETRLELREMISHEQESVLKKLSKDGSTEAGESSHEEDTDGHVAAGSTLARRKRSAGAGSHCQKTSLRVNFEDIGWDSWIIAPKEYEAYECKGGCFFPLAQDVTPTKHAIVQTLVHLKFPTKVGKACCVPTKLSPISVLYKDDMGVPTLKYHYEGMSVAECGCR

SEQ ID NO: 13 - protein, 426 aa, synthetic construct
  source 1..426: note = BMP-9 varient
MAWVWTLLFLMAAAQSIQAKPLQSWGRGSAGGNAHSPLGVPGGGLPEHTFNLKMFLENVKVDFLRSLNLSGVPSQDKTRVEPPQYMIDLYNRYTSDKSTTPASNIVRSFSMEDAISITATEDFPFQKHILLFNISIPRHEQITRAELRLYVSCQNHVDPSHDLKGSVVIYDVLDGTDAWDSATETKTFLVSQDIQDEGWETLEVSSAVKRWVRSDSTKSKNKLEVTVESHRKGCDTLDISVPPGSRNLPFFVVFSNDHSSGTKETRLELREMISHEQESVLKKLSKDGSTEAGESSHEEDTDGHVAAGSTLARRKRSAGAGSHCQKTSLRVNFEDIGWDSWIIAPKEYEAYECKGGCFFPLADDVTPTKHPIVQTLVHLKFPTKVGKACCVPTKLSPISVLYKDDMGVPTLKYHYEGMSVAECGCR

SEQ ID NO: 14 - protein, 426 aa, synthetic construct
  source 1..426: note = BMP-9 varient
MAWVWTLLFLMAAAQSIQAKPLQSWGRGSAGGNAHSPLGVPGGGLPEHTFNLKMFLENVKVDFLRSLNLSGVPSQDKTRVEPPQYMIDLYNRYTSDKSTTPASNIVRSFSMEDAISITATEDFPFQKHILLFNISIPRHEQITRAELRLYVSCQNHVDPSHDLKGSVVIYDVLDGTDAWDSATETKTFLVSQDIQDEGWETLEVSSAVKRWVRSDSTKSKNKLEVTVESHRKGCDTLDISVPPGSRNLPFFVVFSNDHSSGTKETRLELREMISHEQESVLKKLSKDGSTEAGESSHEEDTDGHVAAGSTLARRKRSAGAGSHCQKTSLRVNFEDIGWDSWIIAPKEYEAYECKGGCFFPLADDVTPTKHARVQTLVHLKFPTKVGKACCVPTKLSPISVLYKDDMGVPTLKYHYEGMSVAECGCR

SEQ ID NO: 15 - protein, 426 aa, synthetic construct
  source 1..426: note = BMP-9 varient
MAWVWTLLFLMAAAQSIQAKPLQSWGRGSAGGNAHSPLGVPGGGLPEHTFNLKMFLENVKVDFLRSLNLSGVPSQDKTRVEPPQYMIDLYNRYTSDKSTTPASNIVRSFSMEDAISITATEDFPFQKHILLFNISIPRHEQITRAELRLYVSCQNHVDPSHDLKGSVVIYDVLDGTDAWDSATETKTFLVSQDIQDEGWETLEVSSAVKRWVRSDSTKSKNKLEVTVESHRKGCDTLDISVPPGSRNLPFFVVFSNDHSSGTKETRLELREMISHEQESVLKKLSKDGSTEAGESSHEEDTDGHVAAGSTLARRKRSAGAGSHCQKTSLRVNFEDIGWDSWIIAPKEYEAYECKGGCFFPLADDVTPTKHAIVQTRVHLKFPTKVGKACCVPTKLSPISVLYKDDMGVPTLKYHYEGMSVAECGCR

SEQ ID NO: 16 - protein, 426 aa, synthetic construct
  source 1..426: note = BMP-9 varient
MAWVWTLLFLMAAAQSIQAKPLQSWGRGSAGGNAHSPLGVPGGGLPEHTFNLKMFLENVKVDFLRSLNLSGVPSQDKTRVEPPQYMIDLYNRYTSDKSTTPASNIVRSFSMEDAISITATEDFPFQKHILLFNISIPRHEQITRAELRLYVSCQNHVDPSHDLKGSVVIYDVLDGTDAWDSATETKTFLVSQDIQDEGWETLEVSSAVKRWVRSDSTKSKNKLEVTVESHRKGCDTLDISVPPGSRNLPFFVVFSNDHSSGTKETRLELREMISHEQESVLKKLSKDGSTEAGESSHEEDTDGHVAAGSTLARRKRSAGAGSHCQKTSLRVNFEDIGWDSWIIAPKEYEAYECKGGCFFPLADDVTPTKHHKVQTLVHLKFPTKVGKACCVPTKLSPISVLYKDDMGVPTLKYHYEGMSVAECGCR

SEQ ID NO: 17 - protein, 426 aa, synthetic construct
  source 1..426: note = BMP-9 varient
MAWVWTLLFLMAAAQSIQAKPLQSWGRGSAGGNAHSPLGVPGGGLPEHTFNLKMFLENVKVDFLRSLNLSGVPSQDKTRVEPPQYMIDLYNRYTSDKSTTPASNIVRSFSMEDAISITATEDFPFQKHILLFNISIPRHEQITRAELRLYVSCQNHVDPSHDLKGSVVIYDVLDGTDAWDSATETKTFLVSQDIQDEGWETLEVSSAVKRWVRSDSTKSKNKLEVTVESHRKGCDTLDISVPPGSRNLPFFVVFSNDHSSGTKETRLELREMISHEQESVLKKLSKDGSTEAGESSHEEDTDGHVAAGSTLARRKRSAGAGSHCQKTSLRVNFEDIGWDSWIIAPKEYEAYECKGGCFFPLADDVTPTKRRKVQTLVHLKFPTKVGKACCVPTKLSPISVLYKDDMGVPTLKYHYEGMSVAECGCR

SEQ ID NO: 18 - protein, 426 aa, synthetic construct
  source 1..426: note = BMP-9 varient
MAWVWTLLFLMAAAQSIQAKPLQSWGRGSAGGNAHSPLGVPGGGLPEHTFNLKMFLENVKVDFLRSLNLSGVPSQDKTRVEPPQYMIDLYNRYTSDKSTTPASNIVRSFSMEDAISITATEDFPFQKHILLFNISIPRHEQITRAELRLYVSCQNHVDPSHDLKGSVVIYDVLDGTDAWDSATETKTFLVSQDIQDEGWETLEVSSAVKRWVRSDSTKSKNKLEVTVESHRKGCDTLDISVPPGSRNLPFFVVFSNDHSSGTKETRLELREMISHEQESVLKKLSKDGSTEAGESSHEEDTDGHVAAGSTLARRKRSAGAGSHCQKTSLRVNFEDIGWDSWIIAPKEYEAYECKGGCFFPLADDVTPTKHRKVRTRVHLKFPTKVGKACCVPTKLSPISVLYKDDMGVPTLKYHYEGMSVAECGCR

SEQ ID NO: 19 - protein, 426 aa, synthetic construct
  source 1..426: note = BMP-9 varient
MAWVWTLLFLMAAAQSIQAKPLQSWGRGSAGGNAHSPLGVPGGGLPEHTFNLKMFLENVKVDFLRSLNLSGVPSQDKTRVEPPQYMIDLYNRYTSDKSTTPASNIVRSFSMEDAISITATEDFPFQKHILLFNISIPRHEQITRAELRLYVSCQNHVDPSHDLKGSVVIYDVLDGTDAWDSATETKTFLVSQDIQDEGWETLEVSSAVKRWVRSDSTKSKNKLEVTVESHRKGCDTLDISVPPGSRNLPFFVVFSNDHSSGTKETRLELREMISHEQESVLKKLSKDGSTEAGESSHEEDTDGHVAAGSTLARRKRSAGAGSHCQKTSLRVNFEDIGWDSWIIAPKEYEAYECKGGCFFPLADDVTPTKPRIVQTLVHLKFPTKVGKACCVPTKLSPISVLYKDDMGVPTLKYHYEGMSVAECGCR

SEQ ID NO: 20 - protein, 426 aa, synthetic construct
  source 1..426: note = BMP-9 varient
MAWVWTLLFLMAAAQSIQAKPLQSWGRGSAGGNAHSPLGVPGGGLPEHTFNLKMFLENVKVDFLRSLNLSGVPSQDKTRVEPPQYMIDLYNRYTSDKSTTPASNIVRSFSMEDAISITATEDFPFQKHILLFNISIPRHEQITRAELRLYVSCQNHVDPSHDLKGSVVIYDVLDGTDAWDSATETKTFLVSQDIQDEGWETLEVSSAVKRWVRSDSTKSKNKLEVTVESHRKGCDTLDISVPPGSRNLPFFVVFSNDHSSGTKETRLELREMISHEQESVLKKLSKDGSTEAGESSHEEDTDGHVAAGSTLARRKRSAGAGSHCQKTSLRVNFEDIGWDSWIIAPKEYEAYECKGGCFWPLADDVTPTKHAIVQTLVHLKYPTKVGKACCVPTKLSPISVLYKDDMGVPTLKYHYEGMSVAECGCR

SEQ ID NO: 21 - protein, 426 aa, synthetic construct
  source 1..426: note = BMP-9 varient
MAWVWTLLFLMAAAQSIQAKPLQSWGRGSAGGNAHSPLGVPGGGLPEHTFNLKMFLENVKVDFLRSLNLSGVPSQDKTRVEPPQYMIDLYNRYTSDKSTTPASNIVRSFSMEDAISITATEDFPFQKHILLFNISIPRHEQITRAELRLYVSCQNHVDPSHDLKGSVVIYDVLDGTDAWDSATETKTFLVSQDIQDEGWETLEVSSAVKRWVRSDSTKSKNKLEVTVESHRKGCDTLDISVPPGSRNLPFFVVFSNDHSSGTKETRLELREMISHEQESVLKKLSKDGSTEAGESSHEEDTDGHVAAGSTLARRKRSAGAGSHCQKTSLRVNFEDIGWDSWIIAPKEYEAYECKGGCFFPCADDVTPTKHCIDQTLDHLKFPTKVGKACCVPTKLSPISVLYKDDMGVPTLKYHYEGMSVAECGCR

SEQ ID NO: 22 - protein, 426 aa, synthetic construct
  source 1..426: note = BMP-9 varient
MAWVWTLLFLMAAAQSIQAKPLQSWGRGSAGGNAHSPLGVPGGGLPEHTFNLKMFLENVKVDFLRSLNLSGVPSQDKTRVEPPQYMIDLYNRYTSDKSTTPASNIVRSFSMEDAISITATEDFPFQKHILLFNISIPRHEQITRAELRLYVSCQNHVDPSHDLKGSVVIYDVLDGTDAWDSATETKTFLVSQDIQDEGWETLEVSSAVKRWVRSDSTKSKNKLEVTVESHRKGCDTLDISVPPGSRNLPFFVVFSNDHSSGTKETRLELREMISHEQESVLKKLSKDGSTEAGESSHEEDTDGHVAAGSTLARRKRSAGAGSHCQKTSLRVNFEDIGWDSWIIAPKEYEAYECKGGCFFPLADDVTPTKHAIVQTLVHLKCGGKVGKACCVPTKLSPISVLYKDDMGVPTLKYHYEGMSVAECGCR

SEQ ID NO: 23 - protein, 426 aa, synthetic construct
  source 1..426: note = BMP-9 varient
MAWVWTLLFLMAAAQSIQAKPLQSWGRGSAGGNAHSPLGVPGGGLPEHTFNLKMFLENVKVDFLRSLNLSGVPSQDKTRVEPPQYMIDLYNRYTSDKSTTPASNIVRSFSMEDAISITATEDFPFQKHILLFNISIPRHEQITRAELRLYVSCQNHVDPSHDLKGSVVIYDVLDGTDAWDSATETKTFLVSQDIQDEGWETLEVSSAVKRWVRSDSTKSKNKLEVTVESHRKGCDTLDISVPPGSRNLPFFVVFSNDHSSGTKETRLELREMISHEQESVLKKLSKDGSTEAGESSHEEDTDGHVAAGSTLARRKRSAGAGSHCQKTSLRVNFEDIGWDSWIIAPKEYEAYECKGGCFFPCADDVTPTKHCIDQTLDHLKFPTKVGKDCCVPTKISPISVLWKDDMGVPTLKYHYEGMSVAECGCR

SEQ ID NO: 24 - protein, 426 aa, synthetic construct
  source 1..426: note = BMP-9 varient
MAWVWTLLFLMAAAQSIQAKPLQSWGRGSAGGNAHSPLGVPGGGLPEHTFNLKMFLENVKVDFLRSLNLSGVPSQDKTRVEPPQYMIDLYNRYTSDKSTTPASNIVRSFSMEDAISITATEDFPFQKHILLFNISIPRHEQITRAELRLYVSCQNHVDPSHDLKGSVVIYDVLDGTDAWDSATETKTFLVSQDIQDEGWETLEVSSAVKRWVRSDSTKSKNKLEVTVESHRKGCDTLDISVPPGSRNLPFFVVFSNDHSSGTKETRLELREMISHEQESVLKKLSKDGSTEAGESSHEEDTDGHVAAGSTLARRKRSAGAGSHCQKTSLRVNFEDIGWDSWIIAPKEYEAYECKGGCFFPLADDVTPTKHAIVQTLVHLKCGGKVGKACCAPTPLSPISVLWKDDMGVPTLKYHYEGMSVAECGCR

SEQ ID NO: 25 - protein, 426 aa, synthetic construct
  source 1..426: note = BMP-9 varient
MAWVWTLLFLMAAAQSIQAKPLQSWGRGSAGGNAHSPLGVPGGGLPEHTFNLKMFLENVKVDFLRSLNLSGVPSQDKTRVEPPQYMIDLYNRYTSDKSTTPASNIVRSFSMEDAISITATEDFPFQKHILLFNISIPRHEQITRAELRLYVSCQNHVDPSHDLKGSVVIYDVLDGTDAWDSATETKTFLVSQDIQDEGWETLEVSSAVKRWVRSDSTKSKNKLEVTVESHRKGCDTLDISVPPGSRNLPFFVVFSNDHSSGTKETRLELREMISHEQESVLKKLSKDGSTEAGESSHEEDTDGHVAAGSTLARRKRSAGAGSHCQKTSLRVNFEDIGWDSWIIAPKEYEAYECKGGCFFPLAADVTPTKHAIVQTLVHLKFPTKVGKACCVPTKLSPISVLYKDDMGVPTLKYHYEGMSVAECGCR

SEQ ID NO: 26 - protein, 426 aa, synthetic construct
  source 1..426: note = BMP-9 varient
MAWVWTLLFLMAAAQSIQAKPLQSWGRGSAGGNAHSPLGVPGGGLPEHTFNLKMFLENVKVDFLRSLNLSGVPSQDKTRVEPPQYMIDLYNRYTSDKSTTPASNIVRSFSMEDAISITATEDFPFQKHILLFNISIPRHEQITRAELRLYVSCQNHVDPSHDLKGSVVIYDVLDGTDAWDSATETKTFLVSQDIQDEGWETLEVSSAVKRWVRSDSTKSKNKLEVTVESHRKGCDTLDISVPPGSRNLPFFVVFSNDHSSGTKETRLELREMISHEQESVLKKLSKDGSTEAGESSHEEDTDGHVAAGSTLARRKRSAGAGSHCQKTSLRVNFEDIGWDSWIIAPKEYEAYECKGGCFFPLADDVTPTKHAIVQTLVHLKFPTKVGKACCVPTKLSPISVLYKDAMGVPTLKYHYEGMSVAECGCR

SEQ ID NO: 27 - protein, 426 aa, synthetic construct
  source 1..426: note = BMP-9 varient
MAWVWTLLFLMAAAQSIQAKPLQSWGRGSAGGNAHSPLGVPGGGLPEHTFNLKMFLENVKVDFLRSLNLSGVPSQDKTRVEPPQYMIDLYNRYTSDKSTTPASNIVRSFSMEDAISITATEDFPFQKHILLFNISIPRHEQITRAELRLYVSCQNHVDPSHDLKGSVVIYDVLDGTDAWDSATETKTFLVSQDIQDEGWETLEVSSAVKRWVRSDSTKSKNKLEVTVESHRKGCDTLDISVPPGSRNLPFFVVFSNDHSSGTKETRLELREMISHEQESVLKKLSKDGSTEAGESSHEEDTDGHVAAGSTLARRKRSAGAGSHCQKTSLRVNFEDIGWDSWIIAPKEYEAYECKGGCFFPLAEDVTPTKHAIVQTLVHLKFPTKVGKACCVPTKLSPISVLYKDDMGVPTLKYHYEGMSVAECGCR

SEQ ID NO: 28 - protein, 426 aa, synthetic construct
  source 1..426: note = BMP-9 varient
MAWVWTLLFLMAAAQSIQAKPLQSWGRGSAGGNAHSPLGVPGGGLPEHTFNLKMFLENVKVDFLRSLNLSGVPSQDKTRVEPPQYMIDLYNRYTSDKSTTPASNIVRSFSMEDAISITATEDFPFQKHILLFNISIPRHEQITRAELRLYVSCQNHVDPSHDLKGSVVIYDVLDGTDAWDSATETKTFLVSQDIQDEGWETLEVSSAVKRWVRSDSTKSKNKLEVTVESHRKGCDTLDISVPPGSRNLPFFVVFSNDHSSGTKETRLELREMISHEQESVLKKLSKDGSTEAGESSHEEDTDGHVAAGSTLARRKRSAGAGSHCQKTSLRVNFEDIGWDSWIIAPKEYEAYECKGGCFFPLAADVTPTKHAIVQTLVHLKFPTKVGKACCVPTKLSPISVLYKDAMGVPTLKYHYEGMSVAECGCR

SEQ ID NO: 29 - protein, 24 aa, synthetic construct
  source 1..24: note = BMP-9 varient
FFPLADDVTPTKHAIVQTLVHLKF

SEQ ID NO: 30 - protein, 243 aa, synthetic construct
  source 1..243: note = Fc
MAWVWTLLFLMAAAQSIQAHTCPPCPAPELLGGPSVFLFPPKPKDTLMISRTPEVTCVVVDVSHEDPEVKFNWYVDGVEVHNAKTKPREEQYNSTYRVVSVLTVLHQDWLNGKEYKCKVSNKALPAPIEKTISKAKGQPREPQVYTLPPSRDELTKNQVSLTCLVKGFYPSDIAVEWESNGQPENNYKTTPPVLDSDGSFFLYSKLTVDKSRWQQGNVFSCSVMHEALHNHYTQKSLSLSPGK

SEQ ID NO: 31 - protein, 15 aa, synthetic construct
  source 1..15: note = Linker
GGGGSGGGGSGGGGS

SEQ ID NO: 32 - protein, 368 aa, synthetic construct
  source 1..368: note = BMP-Fc fusion
MAWVWTLLFLMAAAQSIQAHTCPPCPAPELLGGPSVFLFPPKPKDTLMISRTPEVTCVVVDVSHEDPEVKFNWYVDGVEVHNAKTKPREEQYNSTYRVVSVLTVLHQDWLNGKEYKCKVSNKALPAPIEKTISKAKGQPREPQVYTLPPSRDELTKNQVSLTCLVKGFYPSDIAVEWESNGQPENNYKTTPPVLDSDGSFFLYSKLTVDKSRWQQGNVFSCSVMHEALHNHYTQKSLSLSPGKGGGGSGGGGSGGGGSSAGAGSHCQKTSLRVNFEDIGWDSWIIAPKEYEAYECKGGCFFPLADDVTPTKHAIVQTLVHLKFPTKVGKACCVPTKLSPISVLYKDDMGVPTLKYHYEGMSVAECGCR

SEQ ID NO: 33 - protein, 665 aa, synthetic construct
  source 1..665: note = BMP-Fc fusion
MAWVWTLLFLMAAAQSIQAKPLQSWGRGSAGGNAHSPLGVPGGGLPEHTFNLKMFLENVKVDFLRSLNLSGVPSQDKTRVEPPQYMIDLYNRYTSDKSTTPASNIVRSFSMEDAISITATEDFPFQKHILLFNISIPRHEQITRAELRLYVSCQNHVDPSHDLKGSVVIYDVLDGTDAWDSATETKTFLVSQDIQDEGWETLEVSSAVKRWVRSDSTKSKNKLEVTVESHRKGCDTLDISVPPGSRNLPFFVVFSNDHSSGTKETRLELREMISHEQESVLKKLSKDGSTEAGESSHEEDTDGHVAAGSTLARRKRSAGAGSHCQKTSLRVNFEDIGWDSWIIAPKEYEAYECKGGCFFPLADDVTPTKHAIVQTLVHLKFPTKVGKACCVPTKLSPISVLYKDDMGVPTLKYHYEGMSVAECGCRGGGGSGGGGSGGGGSHTCPPCPAPELLGGPSVFLFPPKPKDTLMISRTPEVTCVVVDVSHEDPEVKFNWYVDGVEVHNAKTKPREEQYNSTYRVVSVLTVLHQDWLNGKEYKCKVSNKALPAPIEKTISKAKGQPREPQVYTLPPSRDELTKNQVSLTCLVKGFYPSDIAVEWESNGQPENNYKTTPPVLDSDGSFFLYSKLTVDKSRWQQGNVFSCSVMHEALHNHYTQKSLSLSPGK

SEQ ID NO: 34 - protein, 20 aa, synthetic construct
KVGKACCVPTKLSPISVLYK